European Patent Application EP 4 365 295 A1, published May 8, 2024. Title: Chimeric cytokine receptor. Applicant: Aichi Prefecture. The sequence listing filed with the application follows.

SEQUENCE LISTING (36 sequences)

SEQ ID NO: 1 - protein, 459 aa, Homo sapiens
MTILGTTFGMVFSLLQVVSGESGYAQNGDLEDAELDDYSFSCYSQLEVNGSQHSLTCAFEDPDVNITNLEFEICGALVEVKCLNFRKLQEIYFIETKKFLLIGKSNICVKVGEKSLTCKKIDLTTIVKPEAPFDLSVVYREGANDFVVTFNTSHLQKKYVKVLMHDVAYRQEKDENKWTHVNLSSTKLTLLQRKLQPAAMYEIKVRSIPDHYFKGFWSEWSPSYYFRTPEINNSSGEMDPILLTISILSFFSVALLVILACVLWKKRIKPIVWPSLPDHKKTLEHLCKKPRKNLNVSFNPESFLDCQIHRVDDIQARDEVEGFLQDTFPQQLEESEKQRLGGDVQSPNCPSEDVVITPESFGRDSSLTCLAGNVSACDAPILSSSRSLDCRESGKNGPHVYQDLLLSLGTTNSTLPPPFSLQSGILTLNPVAQGQPILTSLGSNQEEAYVTMSSFYQNQ

SEQ ID NO: 2 - protein, 4 aa, Homo sapiens
PPCL

SEQ ID NO: 3 - protein, 5 aa, Homo sapiens
FSCGP

SEQ ID NO: 4 - protein, 3 aa, Homo sapiens
CHL

SEQ ID NO: 5 - protein, 7 aa, Homo sapiens
PPVCSVT

SEQ ID NO: 6 - protein, 3 aa, Homo sapiens
KCH

SEQ ID NO: 7 - protein, 569 aa, Homo sapiens
MKVLLRLICFIALLISSLEADKCKEREEKIILVSSANEIDVRPCPLNPNEHKGTITWYKDDSKTPVSTEQASRIHQHKEKLWFVPAKVEDSGHYYCVVRNSSYCLRIKISAKFVENEPNLCYNAQAIFKQKLPVAGDGGLVCPYMEFFKNENNELPKLQWYKDCKPLLLDNIHFSGVKDRLIVMNVAEKHRGNYTCHASYTYLGKQYPITRVIEFITLEENKPTRPVIVSPANETMEVDLGSQIQLICNVTGQLSDIAYWKWNGSVIDEDDPVLGEDYYSVENPANKRRSTLITVLNISEIESRFYKHPFTCFAKNTHGIDAAYIQLIYPVTNFQKHMIGICVTLTVIIVCSVFIYKIFKIDIVLWYRDSCYDFLPIKASDGKTYDAYILYPKTVGEGSTSDCDIFVFKVLPEVLEKQCGYKLFIYGRDDYVGEDIVEVINENVKKSRRLIIILVRETSGFSWLGGSSEEQIAMYNALVQDGIKVVLLELEKIQDYEKMPESIKFIKQKHGAIRWSGDFTQGPQSAKTRFWKNVRYHMPVQRRSPSSKHQLLSPATKEKLQREAHVPLG

SEQ ID NO: 8 - DNA, 1710 bp, Homo sapiens
atgaaagtgttactcagacttatttgtttcatagctctactgatttcttctctggaggctgataaatgcaaggaacgtgaagaaaaaataattttagtgtcatctgcaaatgaaattgatgttcgtccctgtcctcttaacccaaatgaacacaaaggcactataacttggtataaagatgacagcaagacacctgtatctacagaacaagcctccaggattcatcaacacaaagagaaactttggtttgttcctgctaaggtggaggattcaggacattactattgcgtggtaagaaattcatcttactgcctcagaattaaaataagtgcaaaatttgtggagaatgagcctaacttatgttataatgcacaagccatatttaagcagaaactacccgttgcaggagacggaggacttgtgtgcccttatatggagttttttaaaaatgaaaataatgagttacctaaattacagtggtataaggattgcaaacctctacttcttgacaatatacactttagtggagtcaaagataggctcatcgtgatgaatgtggctgaaaagcatagagggaactatacttgtcatgcatcctacacatacttgggcaagcaatatcctattacccgggtaatagaatttattactctagaggaaaacaaacccacaaggcctgtgattgtgagcccagctaatgagacaatggaagtagacttgggatcccagatacaattgatctgtaatgtcaccggccagttgagtgacattgcttactggaagtggaatgggtcagtaattgatgaagatgacccagtgctaggggaagactattacagtgtggaaaatcctgcaaacaaaagaaggagtaccctcatcacagtgcttaatatatcggaaattgaaagtagattttataaacatccatttacctgttttgccaagaatacacatggtatagatgcagcatatatccagttaatatatccagtcactaatttccagaagcacatgattggtatatgtgtcacgttgacagtcataattgtgtgttctgttttcatctataaaatcttcaagattgacattgtgctttggtacagggattcctgctatgattttctcccaataaaagcttcagatggaaagacctatgacgcatatatactgtatccaaagactgttggggaagggtctacctctgactgtgatatttttgtgtttaaagtcttgcctgaggtcttggaaaaacagtgtggatataagctgttcatttatggaagggatgactacgttggggaagacattgttgaggtcattaatgaaaacgtaaagaaaagcagaagactgattatcattttagtcagagaaacatcaggcttcagctggctgggtggttcatctgaagagcaaatagccatgtataatgctcttgttcaggatggaattaaagttgtcctgcttgagctggagaaaatccaagactatgagaaaatgccagaatcgattaaattcattaagcagaaacatggggctatccgctggtcaggggactttacacagggaccacagtctgcaaagacaaggttctggaagaatgtcaggtaccacatgccagtccagcgacggtcaccttcatctaaacaccagttactgtcaccagccactaaggagaaactgcaaagagaggctcacgtgcctctcgggtag

SEQ ID NO: 9 - protein, 398 aa, Homo sapiens
MLRLYVLVMGVSAFTLQPAAHTGAARSCRFRGRHYKREFRLEGEPVALRCPQVPYWLWASVSPRINLTWHKNDSARTVPGEEETRMWAQDGALWLLPALQEDSGTYVCTTRNASYCDKMSIELRVFENTDAFLPFISYPQILTLSTSGVLVCPDLSEFTRDKTDVKIQWYKDSLLLDKDNEKFLSVRGTTHLLVHDVALEDAGYYRCVLTFAHEGQQYNITRSIELRIKKKKEETIPVIISPLKTISASLGSRLTIPCKVFLGTGTPLTTMLWWTANDTHIESAYPGGRVTEGPRQEYSENNENYIEVPLIFDPVTREDLHMDFKCVVHNTLSFQTLRTTVKEASSTFSWGIVLAPLSLAFLVLGGIWMHRRCKHRTGKADGLTVLWPHHQDFQSYPK

SEQ ID NO: 10 - DNA, 1197 bp, Homo sapiens
atgttgcgcttgtacgtgttggtaatgggagtttctgccttcacccttcagcctgcggcacacacaggggctgccagaagctgccggtttcgtgggaggcattacaagcgggagttcaggctggaaggggagcctgtagccctgaggtgcccccaggtgccctactggttgtgggcctctgtcagcccccgcatcaacctgacatggcataaaaatgactctgctaggacggtcccaggagaagaagagacacggatgtgggcccaggacggtgctctgtggcttctgccagccttgcaggaggactctggcacctacgtctgcactactagaaatgcttcttactgtgacaaaatgtccattgagctcagagtttttgagaatacagatgctttcctgccgttcatctcatacccgcaaattttaaccttgtcaacctctggggtattagtatgccctgacctgagtgaattcacccgtgacaaaactgacgtgaagattcaatggtacaaggattctcttcttttggataaagacaatgagaaatttctaagtgtgagggggaccactcacttactcgtacacgatgtggccctggaagatgctggctattaccgctgtgtcctgacatttgcccatgaaggccagcaatacaacatcactaggagtattgagctacgcatcaagaaaaaaaaagaagagaccattcctgtgatcatttcccccctcaagaccatatcagcttctctggggtcaagactgacaatcccgtgtaaggtgtttctgggaaccggcacacccttaaccaccatgctgtggtggacggccaatgacacccacatagagagcgcctacccgggaggccgcgtgaccgaggggccacgccaggaatattcagaaaataatgagaactacattgaagtgccattgatttttgatcctgtcacaagagaggatttgcacatggattttaaatgtgttgtccataataccctgagttttcagacactacgcaccacagtcaaggaagcctcctccacgttctcctggggcattgtgctggccccactttcactggccttcttggttttggggggaatatggatgcacagacggtgcaaacacagaactggaaaagcagatggtctgactgtgctatggcctcatcatcaagactttcaatcctatcccaagtga

SEQ ID NO: 11 - protein, 468 aa, Homo sapiens
MLAVGCALLAALLAAPGAALAPRRCPAQEVARGVLTSLPGDSVTLTCPGVEPEDNATVHWVLRKPAAGSHPSRWAGMGRRLLLRSVQLHDSGNYSCYRAGRPAGTVHLLVDVPPEEPQLSCFRKSPLSNVVCEWGPRSTPSLTTKAVLLVRKFQNSPAEDFQEPCQYSQESQKFSCQLAVPEGDSSFYIVSMCVASSVGSKFSKTQTFQGCGILQPDPPANITVTAVARNPRWLSVTWQDPHSWNSSFYRLRFELRYRAERSKTFTTWMVKDLQHHCVIHDAWSGLRHVVQLRAQEEFGQGEWSEWSPEAMGTPWTESRSPPAENEVSTPMQALTTNKDDDNILFRDSANATSLPVQDSSSVPLPTFLVAGGSLAFGTLLCIAIVLRFKKTWKLRALKEGKTSMHPPYSLGQLVPERPRPTPVLVPLISPPVSPSSLGSDNTSSHNRPDARDPRSPYDISNTDYFFPR

SEQ ID NO: 12 - DNA, 1407 bp, Homo sapiens
atgctggccgtcggctgcgcgctgctggctgccctgctggccgcgccgggagcggcgctggccccaaggcgctgccctgcgcaggaggtggcgagaggcgtgctgaccagtctgccaggagacagcgtgactctgacctgcccgggggtagagccggaagacaatgccactgttcactgggtgctcaggaagccggctgcaggctcccaccccagcagatgggctggcatgggaaggaggctgctgctgaggtcggtgcagctccacgactctggaaactattcatgctaccgggccggccgcccagctgggactgtgcacttgctggtggatgttccccccgaggagccccagctctcctgcttccggaagagccccctcagcaatgttgtttgtgagtggggtcctcggagcaccccatccctgacgacaaaggctgtgctcttggtgaggaagtttcagaacagtccggccgaagacttccaggagccgtgccagtattcccaggagtcccagaagttctcctgccagttagcagtcccggagggagacagctctttctacatagtgtccatgtgcgtcgccagtagtgtcgggagcaagttcagcaaaactcaaacctttcagggttgtggaatcttgcagcctgatccgcctgccaacatcacagtcactgccgtggccagaaacccccgctggctcagtgtcacctggcaagacccccactcctggaactcatctttctacagactacggtttgagctcagatatcgggctgaacggtcaaagacattcacaacatggatggtcaaggacctccagcatcactgtgtcatccacgacgcctggagcggcctgaggcacgtggtgcagcttcgtgcccaggaggagttcgggcaaggcgagtggagcgagtggagcccggaggccatgggcacgccttggacagaatccaggagtcctccagctgagaacgaggtgtccacccccatgcaggcacttactactaataaagacgatgataatattctcttcagagattctgcaaatgcgacaagcctcccagtgcaagattcttcttcagtaccactgcccacattcctggttgctggagggagcctggccttcggaacgctcctctgcattgccattgttctgaggttcaagaagacgtggaagctgcgggctctgaaggaaggcaagacaagcatgcatccgccgtactctttggggcagctggtcccggagaggcctcgacccaccccagtgcttgttcctctcatctccccaccggtgtcccccagcagcctggggtctgacaatacctcgagccacaaccgaccagatgccagggacccacggagcccttatgacatcagcaatacagactacttcttccccagatag

SEQ ID NO: 13 - protein, 918 aa, Homo sapiens
MLTLQTWLVQALFIFLTTESTGELLDPCGYISPESPVVQLHSNFTAVCVLKEKCMDYFHVNANYIVWKTNHFTIPKEQYTIINRTASSVTFTDIASLNIQLTCNILTFGQLEQNVYGITIISGLPPEKPKNLSCIVNEGKKMRCEWDGGRETHLETNFTLKSEWATHKFADCKAKRDTPTSCTVDYSTVYFVNIEVWVEAENALGKVTSDHINFDPVYKVKPNPPHNLSVINSEELSSILKLTWTNPSIKSVIILKYNIQYRTKDASTWSQIPPEDTASTRSSFTVQDLKPFTEYVFRIRCMKEDGKGYWSDWSEEASGITYEDRPSKAPSFWYKIDPSHTQGYRTVQLVWKTLPPFEANGKILDYEVTLTRWKSHLQNYTVNATKLTVNLTNDRYLATLTVRNLVGKSDAAVLTIPACDFQATHPVMDLKAFPKDNMLWVEWTTPRESVKKYILEWCVLSDKAPCITDWQQEDGTVHRTYLRGNLAESKCYLITVTPVYADGPGSPESIKAYLKQAPPSKGPTVRTKKVGKNEAVLEWDQLPVDVQNGFIRNYTIFYRTIIGNETAVNVDSSHTEYTLSSLTSDTLYMVRMAAYTDEGGKDGPEFTFTTPKFAQGEIEAIVVPVCLAFLLTTLLGVLFCFNKRDLIKKHIWPNVPDPSKSHIAQWSPHTPPRHNFNSKDQMYSDGNFTDVSVVEIEANDKKPFPEDLKSLDLFKKEKINTEGHSSGIGGSSCMSSSRPSISSSDENESSQNTSSTVQYSTVVHSGYRHQVPSVQVFSRSESTQPLLDSEERPEDLQLVDHVDGGDGILPRQQYFKQNCSQHESSPDISHFERSKQVSSVNEEDFVRLKQQISDHISQSCGSGQMKMFQEVSAADAFGPGTEGQVERFETVGMEAATDEGMPKSYLPQTVRQGGYMPQ

SEQ ID NO: 14 - DNA, 2757 bp, Homo sapiens
atgttgacgttgcagacttggctagtgcaagccttgtttattttcctcaccactgaatctacaggtgaacttctagatccatgtggttatatcagtcctgaatctccagttgtacaacttcattctaatttcactgcagtttgtgtgctaaaggaaaaatgtatggattattttcatgtaaatgctaattacattgtctggaaaacaaaccattttactattcctaaggagcaatatactatcataaacagaacagcatccagtgtcacctttacagatatagcttcattaaatattcagctcacttgcaacattcttacattcggacagcttgaacagaatgtttatggaatcacaataatttcaggcttgcctccagaaaaacctaaaaatttgagttgcattgtgaacgaggggaagaaaatgaggtgtgagtgggatggtggaagggaaacacacttggagacaaacttcactttaaaatctgaatgggcaacacacaagtttgctgattgcaaagcaaaacgtgacacccccacctcatgcactgttgattattctactgtgtattttgtcaacattgaagtctgggtagaagcagagaatgcccttgggaaggttacatcagatcatatcaattttgatcctgtatataaagtgaagcccaatccgccacataatttatcagtgatcaactcagaggaactgtctagtatcttaaaattgacatggaccaacccaagtattaagagtgttataatactaaaatataacattcaatataggaccaaagatgcctcaacttggagccagattcctcctgaagacacagcatccacccgatcttcattcactgtccaagaccttaaaccttttacagaatatgtgtttaggattcgctgtatgaaggaagatggtaagggatactggagtgactggagtgaagaagcaagtgggatcacctatgaagatagaccatctaaagcaccaagtttctggtataaaatagatccatcccatactcaaggctacagaactgtacaactcgtgtggaagacattgcctccttttgaagccaatggaaaaatcttggattatgaagtgactctcacaagatggaaatcacatttacaaaattacacagttaatgccacaaaactgacagtaaatctcacaaatgatcgctatctagcaaccctaacagtaagaaatcttgttggcaaatcagatgcagctgttttaactatccctgcctgtgactttcaagctactcaccctgtaatggatcttaaagcattccccaaagataacatgctttgggtggaatggactactccaagggaatctgtaaagaaatatatacttgagtggtgtgtgttatcagataaagcaccctgtatcacagactggcaacaagaagatggtaccgtgcatcgcacctatttaagagggaacttagcagagagcaaatgctatttgataacagttactccagtatatgctgatggaccaggaagccctgaatccataaaggcataccttaaacaagctccaccttccaaaggacctactgttcggacaaaaaaagtagggaaaaacgaagctgtcttagagtgggaccaacttcctgttgatgttcagaatggatttatcagaaattatactatattttatagaaccatcattggaaatgaaactgctgtgaatgtggattcttcccacacagaatatacattgtcctctttgactagtgacacattgtacatggtacgaatggcagcatacacagatgaaggtgggaaggatggtccagaattcacttttactaccccaaagtttgctcaaggagaaattgaagccatagtcgtgcctgtttgcttagcattcctattgacaactcttctgggagtgctgttctgctttaataagcgagacctaattaaaaaacacatctggcctaatgttccagatccttcaaagagtcatattgcccagtggtcacctcacactcctccaaggcacaattttaattcaaaagatcaaatgtattcagatggcaatttcactgatgtaagtgttgtggaaatagaagcaaatgacaaaaagccttttccagaagatctgaaatcattggacctgttcaaaaaggaaaaaattaatactgaaggacacagcagtggtattggggggtcttcatgcatgtcatcttctaggccaagcatttctagcagtgatgaaaatgaatcttcacaaaacacttcgagcactgtccagtattctaccgtggtacacagtggctacagacaccaagttccgtcagtccaagtcttctcaagatccgagtctacccagcccttgttagattcagaggagcggccagaagatctacaattagtagatcatgtagatggcggtgatggtattttgcccaggcaacagtacttcaaacagaactgcagtcagcatgaatccagtccagatatttcacattttgaaaggtcaaagcaagtttcatcagtcaatgaggaagattttgttagacttaaacagcagatttcagatcatatttcacaatcctgtggatctgggcaaatgaaaatgtttcaggaagtttctgcagcagatgcttttggtccaggtactgagggacaagtagaaagatttgaaacagttggcatggaggctgcgactgatgaaggcatgcctaaaagttacttaccacagactgtacggcaaggcggctacatgcctcagtga

SEQ ID NO: 15 - protein, 9 aa, Homo sapiens
VWPSLPDHK

SEQ ID NO: 16 - protein, 4 aa, Homo sapiens
YQNQ

SEQ ID NO: 17 - protein, 4 aa, Homo sapiens
YVTM

SEQ ID NO: 18 - DNA, 2115 bp, Artificial
  synthetic
atgctgaccctgcagacatggctggtgcaggccctgttcatcttcctgaccacagagagcacaggcgagctgctcgatccttgcggctacatctctcctgagagccctgtggtccagctgcacagcaatttcaccgccgtgtgcgtgctgaaagaaaagtgcatggactacttccacgtgaacgccaactacatcgtgtggaaaacgaaccacttcacgatccccaaagagcagtacaccatcatcaaccggaccgccagcagcgtgaccttcacagatatcgccagcctgaacatccagctgacctgcaacatcctgaccttcggccagctggaacagaacgtgtacggcatcacaatcatcagcggcctgcctccagagaagcccaagaacctgagctgcatcgtgaacgagggcaagaaaatgagatgcgagtgggacggcggcagagagacacacctggaaacaaacttcaccctgaagtccgagtgggccacacacaagttcgccgactgcaaggccaagagggatacccctaccagctgtaccgtggactacagcaccgtgtacttcgtgaacatcgaagtgtgggtcgaagccgagaacgccctgggcaaagtgaccagcgaccacatcaacttcgaccccgtgtacaaagtgaagcccaatcctcctcacaacctgagcgtgatcaacagcgaggaactgagcagcatcctgaagctgacatggacaaaccccagcatcaagtccgtgatcatcctcaagtacaacatccagtaccggaccaaggacgccagcacctggtcacagattcctccagaggataccgcctccaccagatccagcttcacagtgcaggacctgaagcctttcaccgagtacgtgttccggatcagatgcatgaaggaagatggcaaaggctactggagcgattggagcgaggaagccagcggcatcacctacgaggatagacctggctctgccggatctgctgctggctctggcgaattcgtggatgtgcctcctgaggaaccccagctgagctgcttcagaaagtcccctctgagcaacgtcgtgtgcgagtggggccctagaagcacacctagcctgacaacaaaggccgtgctgctcgtgcggaagttccagaatagccctgccgaggacttccaagagccttgccagtacagccaagagagccagaagttcagctgtcagctggccgtgcctgagggcgatagcagcttctacatcgtgtctatgtgcgtggccagcagcgtgggcagcaagtttagcaagacccagaccttccaaggctgcggcatcctgcaacctgatcctccagccaacatcaccgtgaccgccgtggccagaaatcccagatggctgtctgtgacctggcaggatccccacagctggaacagcagcttttaccggctgagattcgagctgcggtacagggccgagagaagcaagaccttcaccacctggatggtcaaggacctgcagcaccactgcgtgatccatgacgcttggagcggactgagacacgtggtgcagctgagagcccaagaagagtttggccaaggcgagtggagcgagtggtcacctgaagccatgggcacaccttggaccgagtctagatctccaccagccgagaacgaggtgtccacacctatgcaggccctgaccaccaacaaggacgacgacaacatcctgttccgggacagcgccaatgccacaagtctgcctgtgcaggatagctcctctgtgcctcttcctgcggccgcaattgaagttatgtatcctcctccttacctagacaatgagaagagcaatggaaccattatccatgtgaaagggaaacacctttgtccaagtcccctatttcccggaccttctaagcccttttgggtgctggtggtggttggtggagtcctggcttgctatagcttgctagtaacagtggcctttattattttctgggtgaggagtaagaggagcaggctcctgcacagtgactacatgaacatgcctccccgccgccccgggcccacccgcaagcattaccagccctatgccccaccacgcgacttcgcagcctatcgctcctga

SEQ ID NO: 19 - DNA, 1380 bp, Homo sapiens
atgacaattctaggtacaacttttggcatggttttttctttacttcaagtcgtttctggagaaagtggctatgctcaaaatggagacttggaagatgcagaactggatgactactcattctcatgctatagccagttggaagtgaatggatcgcagcactcactgacctgtgcttttgaggacccagatgtcaacatcaccaatctggaatttgaaatatgtggggccctcgtggaggtaaagtgcctgaatttcaggaaactacaagagatatatttcatcgagacaaagaaattcttactgattggaaagagcaatatatgtgtgaaggttggagaaaagagtctaacctgcaaaaaaatagacctaaccactatagttaaacctgaggctccttttgacctgagtgtcgtctatcgggaaggagccaatgactttgtggtgacatttaatacatcacacttgcaaaagaagtatgtaaaagttttaatgcacgatgtagcttaccgccaggaaaaggatgaaaacaaatggacgcatgtgaatttatccagcacaaagctgacactcctgcagagaaagctccaaccggcagcaatgtatgagattaaagttcgatccatccctgatcactattttaaaggcttctggagtgaatggagtccaagttattacttcagaactccagagatcaataatagctcaggggagatggatcctatcttactaaccatcagcattttgagttttttctctgtcgctctgttggtcatcttggcctgtgtgttatggaaaaaaaggattaagcctatcgtatggcccagtctccccgatcataagaagactctggaacatctttgtaagaaaccaagaaaaaatttaaatgtgagtttcaatcctgaaagtttcctggactgccagattcatagggtggatgacattcaagctagagatgaagtggaaggttttctgcaagatacgtttcctcagcaactagaagaatctgagaagcagaggcttggaggggatgtgcagagccccaactgcccatctgaggatgtagtcatcactccagaaagctttggaagagattcatccctcacatgcctggctgggaatgtcagtgcatgtgacgcccctattctctcctcttccaggtccctagactgcagggagagtggcaagaatgggcctcatgtgtaccaggacctcctgcttagccttgggactacaaacagcacgctgccccctccattttctctccaatctggaatcctgacattgaacccagttgctcagggtcagcccattcttacttccctgggatcaaatcaagaagaagcatatgtcaccatgtccagcttctaccaaaaccagtga

SEQ ID NO: 20 - protein, 400 aa, Homo sapiens
MLLLVTSLLLCELPHPAFLLIPEKSDLRTVAPASSLNVRFDSRTMNLSWDCQENTTFSKCFLTDKKNRVVEPRLSNNECSCTFREICLHEGVTFEVHVNTSQRGFQQKLLYPNSGREGTAAQNFSCFIYNADLMNCTWARGPTAPRDVQYFLYIRNSKRRREIRCPYYIQDSGTHVGCHLDNLSGLTSRNYFLVNGTSREIGIQFFDSLLDTKKIERFNPPSNVTVRCNTTHCLVRWKQPRTYQKLSYLDFQYQLDVHRKNTQPGTENLLINVSGDLENRYNFPSSEPRAKHSVKIRAADVRILNWSSWSEAIEFGSDDGNLGSVYIYVLLIVGTLVCGIVLGFLFKRFLRIQRLFPPVPQIKDKLNDNHEVEDEIIWEEFTPEEGKGYREEVLTVKEIT

SEQ ID NO: 21 - DNA, 1203 bp, Homo sapiens
atgcttctcctggtgacaagccttctgctctgtgagttaccacacccagcattcctcctgatcccagagaaatcggatctgcgaacagtggcaccagcctctagtctcaatgtgaggtttgactccaggacgatgaatttaagctgggactgccaagaaaacacaaccttcagcaagtgtttcttaactgacaagaagaacagagtcgtggaacccaggctcagtaacaacgaatgttcgtgcacatttcgtgaaatttgtctgcatgaaggagtcacatttgaggttcacgtgaatactagtcaaagaggatttcaacagaaactgctttatccaaattcaggaagggagggtaccgctgctcagaatttctcctgtttcatctacaatgcggatttaatgaactgtacctgggcgaggggtccgacggccccccgtgacgtccagtattttttgtacatacgaaactcaaagagaaggagggagatccggtgtccttattacatacaagactcaggaacccatgtgggatgtcacctggataacctgtcaggattaacgtctcgcaattactttctggttaacggaaccagccgagaaattggcatccaattctttgattcacttttggacacaaagaaaatagaacgattcaaccctcccagcaatgtcaccgtacgttgcaacacgacgcactgcctcgtacggtggaaacagcccaggacctatcagaagctgtcgtacctggactttcagtaccagctggacgtccacagaaagaatacccagcctggcacggaaaacctactgattaatgtttctggtgatttggaaaatagatacaactttccaagctctgagcccagagcaaaacacagtgtgaagatcagagctgcagacgtccgcatcttgaattggagctcctggagtgaagccattgaatttggttctgacgacgggaacctcggctctgtgtacatttatgtgctcctaatcgtgggaacccttgtctgtggcatcgtcctcggcttcctctttaaaaggttccttaggatacagcggctgttcccgccagttccacagatcaaagacaaactgaatgataaccatgaggtggaagacgagatcatctgggaggaattcaccccagaggaagggaaaggctaccgcgaagaggtcttgaccgtgaaggaaattacctga

SEQ ID NO: 22 - protein, 897 aa, Homo sapiens
MVLAQGLLSMALLALCWERSLAGAEETIPLQTLRCYNDYTSHITCRWADTQDAQRLVNVTLIRRVNEDLLEPVSCDLSDDMPWSACPHPRCVPRRCVIPCQSFVVTDVDYFSFQPDRPLGTRLTVTLTQHVQPPEPRDLQISTDQDHFLLTWSVALGSPQSHWLSPGDLEFEVVYKRLQDSWEDAAILLSNTSQATLGPEHLMPSSTYVARVRTRLAPGSRLSGRPSKWSPEVCWDSQPGDEAQPQNLECFFDGAAVLSCSWEVRKEVASSVSFGLFYKPSPDAGEEECSPVLREGLGSLHTRHHCQIPVPDPATHGQYIVSVQPRRAEKHIKSSVNIQMAPPSLNVTKDGDSYSLRWETMKMRYEHIDHTFEIQYRKDTATWKDSKTETLQNAHSMALPALEPSTRYWARVRVRTSRTGYNGIWSEWSEARSWDTESVLPMWVLALIVIFLTIAVLLALRFCGIYGYRLRRKWEEKIPNPSKSHLFQNGSAELWPPGSMSAFTSGSPPHQGPWGSRFPELEGVFPVGFGDSEVSPLTIEDPKHVCDPPSGPDTTPAASDLPTEQPPSPQPGPPAASHTPEKQASSFDFNGPYLGPPHSRSLPDILGQPEPPQEGGSQKSPPPGSLEYLCLPAGGQVQLVPLAQAMGPGQAVEVERRPSQGAAGSPSLESGGGPAPPALGPRVGGQDQKDSPVAIPMSSGDTEDPGVASGYVSSADLVFTPNSGASSVSLVPSLGLPSDQTPSLCPGLASGPPGAPGPVKSGFEGYVELPPIEGRSPRSPRNNPVPPEAKSPVLNPGERPADVSPTSPQPEGLLVLQQVGDYCFLPGLGPGPLSLRSKPSSPGPGPEIKNLDQAFQVKKPPGQAVPQVPVIQLFKALKQQDYLSLPPWEVNKPGEVC

SEQ ID NO: 23 - DNA, 2694 bp, Homo sapiens
atggtgctggcccaggggctgctctccatggccctgctggccctgtgctgggagcgcagcctggcaggggcagaagaaaccatcccgctgcagaccctgcgctgctacaacgactacaccagccacatcacctgcaggtgggcagacacccaggatgcccagcggctcgtcaacgtgaccctcattcgccgggtgaatgaggacctcctggagccagtgtcctgtgacctcagtgatgacatgccctggtcagcctgcccccatccccgctgcgtgcccaggagatgtgtcattccctgccagagttttgtcgtcactgacgttgactacttctcattccaaccagacaggcctctgggcacccggctcaccgtcactctgacccagcatgtccagcctcctgagcccagggacctgcagatcagcaccgaccaggaccacttcctgctgacctggagtgtggcccttgggagtccccagagccactggttgtccccaggggatctggagtttgaggtggtctacaagcggcttcaggactcttgggaggacgcagccatcctcctctccaacacctcccaggccaccctggggccagagcacctcatgcccagcagcacctacgtggcccgagtacggacccgcctggccccaggttctcggctctcaggacgtcccagcaagtggagcccagaggtttgctgggactcccagccaggggatgaggcccagccccagaacctggagtgcttctttgacggggccgccgtgctcagctgctcctgggaggtgaggaaggaggtggccagctcggtctcctttggcctattctacaagcccagcccagatgcaggggaggaagagtgctccccagtgctgagggaggggctcggcagcctccacaccaggcaccactgccagattcccgtgcccgaccccgcgacccacggccaatacatcgtctctgttcagccaaggagggcagagaaacacataaagagctcagtgaacatccagatggcccctccatccctcaacgtgaccaaggatggagacagctacagcctgcgctgggaaacaatgaaaatgcgatacgaacacatagaccacacatttgagatccagtacaggaaagacacggccacgtggaaggacagcaagaccgagaccctccagaacgcccacagcatggccctgccagccctggagccctccaccaggtactgggccagggtgagggtcaggacctcccgcaccggctacaacgggatctggagcgagtggagtgaggcgcgctcctgggacaccgagtcggtgctgcctatgtgggtgctggccctcatcgtgatcttcctcaccatcgctgtgctcctggccctccgcttctgtggcatctacgggtacaggctgcgcagaaagtgggaggagaagatccccaaccccagcaagagccacctgttccagaacgggagcgcagagctttggcccccaggcagcatgtcggccttcactagcgggagtcccccacaccaggggccgtggggcagccgcttccctgagctggagggggtgttccctgtaggattcggggacagcgaggtgtcacctctcaccatagaggaccccaagcatgtctgtgatccaccatctgggcctgacacgactccagctgcctcagatctacccacagagcagccccccagcccccagccaggcccgcctgccgcctcccacacacctgagaaacaggcttccagctttgacttcaatgggccctacctggggccgccccacagccgctccctacctgacatcctgggccagccggagcccccacaggagggtgggagccagaagtccccacctccagggtccctggagtacctgtgtctgcctgctggggggcaggtgcaactggtccctctggcccaggcgatgggaccaggacaggccgtggaagtggagagaaggccgagccagggggctgcagggagtccctccctggagtccgggggaggccctgcccctcctgctcttgggccaagggtgggaggacaggaccaaaaggacagccctgtggctatacccatgagctctggggacactgaggaccctggagtggcctctggttatgtctcctctgcagacctggtattcaccccaaactcaggggcctcgtctgtctccctagttccctctctgggcctcccctcagaccagacccccagcttatgtcctgggctggccagtggaccccctggagccccaggccctgtgaagtcagggtttgagggctatgtggagctccctccaattgagggccggtcccccaggtcaccaaggaacaatcctgtcccccctgaggccaaaagccctgtcctgaacccaggggaacgcccggcagatgtgtccccaacatccccacagcccgagggcctccttgtcctgcagcaagtgggcgactattgcttcctccccggcctggggcccggccctctctcgctccggagtaaaccttcttccccgggacccggtcctgagatcaagaacctagaccaggcttttcaagtcaagaagcccccaggccaggctgtgccccaggtgcccgtcattcagctcttcaaagccctgaagcagcaggactacctgtctctgcccccttgggaggtcaacaagcctggggaggtgtgttga

SEQ ID NO: 24 - protein, 598 aa, Artificial
  synthetic
MMRPIVLVLLFATSALALAPRRCPAQEVARGVLTSLPGDSVTLTCPGVEPEDNATVHWVLRKPAAGSHPSRWAGMGRRLLLRSVQLHDSGNYSCYRAGRPAGTVHLLVDVPPEEPQLSCFRKSPLSNVVCEWGPRSTPSLTTKAVLLVRKFQNSPAEDFQEPCQYSQESQKFSCQLAVPEGDSSFYIVSMCVASSVGSKFSKTQTFQGCGILQPDPPANITVTAVARNPRWLSVTWQDPHSWNSSFYRLRFELRYRAERSKTFTTWMVKDLQHHCVIHDAWSGLRHVVQLRAQEEFGQGEWSEWSPEAMGTPWTESRSPPAENEVSTPMQALTTNKDDDNILFRDSANATSLPVQDSSSVPLPAAANNSSGEMDPILLPPCLTISILSFFSVALLVILACVLWKKRIKPIVWPSLPDHKKTLEHLCKKPRKNLNVSFNPESFLDCQIHRVDDIQARDEVEGFLQDTFPQQLEESEKQRLGGDVQSPNCPSEDVVITPESFGRDSSLTCLAGNVSACDAPILSSSRSLDCRESGKNGPHVYQDLLLSLGTTNSTLPPPFSLQSGILTLNPVAQGQPILTSLGSNQEEAYVTMSSFYQNQ

SEQ ID NO: 25 - protein, 829 aa, Artificial
  synthetic
MLTLQTWLVQALFIFLTTESTGELLDPCGYISPESPVVQLHSNFTAVCVLKEKCMDYFHVNANYIVWKTNHFTIPKEQYTIINRTASSVTFTDIASLNIQLTCNILTFGQLEQNVYGITIISGLPPEKPKNLSCIVNEGKKMRCEWDGGRETHLETNFTLKSEWATHKFADCKAKRDTPTSCTVDYSTVYFVNIEVWVEAENALGKVTSDHINFDPVYKVKPNPPHNLSVINSEELSSILKLTWTNPSIKSVIILKYNIQYRTKDASTWSQIPPEDTASTRSSFTVQDLKPFTEYVFRIRCMKEDGKGYWSDWSEEASGITYEDRPGSAGSAAGSGEFVDVPPEEPQLSCFRKSPLSNVVCEWGPRSTPSLTTKAVLLVRKFQNSPAEDFQEPCQYSQESQKFSCQLAVPEGDSSFYIVSMCVASSVGSKFSKTQTFQGCGILQPDPPANITVTAVARNPRWLSVTWQDPHSWNSSFYRLRFELRYRAERSKTFTTWMVKDLQHHCVIHDAWSGLRHVVQLRAQEEFGQGEWSEWSPEAMGTPWTESRSPPAENEVSTPMQALTTNKDDDNILFRDSANATSLPVQDSSSVPLPAAANNSSGEMDPILLPPCLTISILSFFSVALLVILACVLWKKRIKPIVWPSLPDHKKTLEHLCKKPRKNLNVSFNPESFLDCQIHRVDDIQARDEVEGFLQDTFPQQLEESEKQRLGGDVQSPNCPSEDVVITPESFGRDSSLTCLAGNVSACDAPILSSSRSLDCRESGKNGPHVYQDLLLSLGTTNSTLPPPFSLQSGILTLNPVAQGQPILTSLGSNQEEAYVTMSSFYQNQ

SEQ ID NO: 26 - protein, 578 aa, Artificial
  synthetic
MLRLYVLVMGVSAFTLQPAAHTGAARSCRFRGRHYKREFRLEGEPVALRCPQVPYWLWASVSPRINLTWHKNDSARTVPGEEETRMWAQDGALWLLPALQEDSGTYVCTTRNASYCDKMSIELRVFENTDAFLPFISYPQILTLSTSGVLVCPDLSEFTRDKTDVKIQWYKDSLLLDKDNEKFLSVRGTTHLLVHDVALEDAGYYRCVLTFAHEGQQYNITRSIELRIKKKKEETIPVIISPLKTISASLGSRLTIPCKVFLGTGTPLTTMLWWTANDTHIESAYPGGRVTEGPRQEYSENNENYIEVPLIFDPVTREDLHMDFKCVVHNTLSFQTLRTTVKEAAANNSSGEMDPILLPPCLTISILSFFSVALLVILACVLWKKRIKPIVWPSLPDHKKTLEHLCKKPRKNLNVSFNPESFLDCQIHRVDDIQARDEVEGFLQDTFPQQLEESEKQRLGGDVQSPNCPSEDVVITPESFGRDSSLTCLAGNVSACDAPILSSSRSLDCRESGKNGPHVYQDLLLSLGTTNSTLPPPFSLQSGILTLNPVAQGQPILTSLGSNQEEAYVTMSSFYQNQ

SEQ ID NO: 27 - protein, 555 aa, Artificial
  synthetic
MLLLVTSLLLCELPHPAFLLIPEKSDLRTVAPASSLNVRFDSRTMNLSWDCQENTTFSKCFLTDKKNRVVEPRLSNNECSCTFREICLHEGVTFEVHVNTSQRGFQQKLLYPNSGREGTAAQNFSCFIYNADLMNCTWARGPTAPRDVQYFLYIRNSKRRREIRCPYYIQDSGTHVGCHLDNLSGLTSRNYFLVNGTSREIGIQFFDSLLDTKKIERFNPPSNVTVRCNTTHCLVRWKQPRTYQKLSYLDFQYQLDVHRKNTQPGTENLLINVSGDLENRYNFPSSEPRAKHSVKIRAADVRILNWSSWSEAIEFGSDDGAAANNSSGEMDPILLPPCLTISILSFFSVALLVILACVLWKKRIKPIVWPSLPDHKKTLEHLCKKPRKNLNVSFNPESFLDCQIHRVDDIQARDEVEGFLQDTFPQQLEESEKQRLGGDVQSPNCPSEDVVITPESFGRDSSLTCLAGNVSACDAPILSSSRSLDCRESGKNGPHVYQDLLLSLGTTNSTLPPPFSLQSGILTLNPVAQGQPILTSLGSNQEEAYVTMSSFYQNQ

SEQ ID NO: 28 - protein, 678 aa, Artificial
  synthetic
MVLAQGLLSMALLALCWERSLAGAEETIPLQTLRCYNDYTSHITCRWADTQDAQRLVNVTLIRRVNEDLLEPVSCDLSDDMPWSACPHPRCVPRRCVIPCQSFVVTDVDYFSFQPDRPLGTRLTVTLTQHVQPPEPRDLQISTDQDHFLLTWSVALGSPQSHWLSPGDLEFEVVYKRLQDSWEDAAILLSNTSQATLGPEHLMPSSTYVARVRTRLAPGSRLSGRPSKWSPEVCWDSQPGDEAQPQNLECFFDGAAVLSCSWEVRKEVASSVSFGLFYKPSPDAGEEECSPVLREGLGSLHTRHHCQIPVPDPATHGQYIVSVQPRRAEKHIKSSVNIQMAPPSLNVTKDGDSYSLRWETMKMRYEHIDHTFEIQYRKDTATWKDSKTETLQNAHSMALPALEPSTRYWARVRVRTSRTGYNGIWSEWSEARSWDTESVLPMWAAANNSSGEMDPILLPPCLTISILSFFSVALLVILACVLWKKRIKPIVWPSLPDHKKTLEHLCKKPRKNLNVSFNPESFLDCQIHRVDDIQARDEVEGFLQDTFPQQLEESEKQRLGGDVQSPNCPSEDVVITPESFGRDSSLTCLAGNVSACDAPILSSSRSLDCRESGKNGPHVYQDLLLSLGTTNSTLPPPFSLQSGILTLNPVAQGQPILTSLGSNQEEAYVTMSSFYQNQ

SEQ ID NO: 29 - DNA, 1797 bp, Artificial
  synthetic
atgatgaggcccatcgtgctggtgctgctgtttgccacatctgccctggctctggcccctagaagatgccctgctcaagaggtggcaagaggcgtgctgacatctctgcctggcgatagcgtgaccctgacatgtcctggcgtggaacccgaggataatgccaccgtgcattgggtgctgagaaagcctgccgccggatctcacccttctagatgggctggcatgggccgtagactgctgctgagatctgtccagctgcacgacagcggcaactacagctgttacagagccggcagacctgccggaacagtgcatctgctggtggatgtgcctcctgaggaaccccagctgagctgcttcagaaagtcccctctgagcaacgtcgtgtgcgagtggggccctagaagcacacctagcctgacaacaaaggccgtgctgctcgtgcggaagttccagaatagccctgccgaggacttccaagagccttgccagtacagccaagagagccagaagttcagctgtcagctggccgtgcctgagggcgatagcagcttctacatcgtgtctatgtgcgtggccagcagcgtgggcagcaagtttagcaagacccagaccttccaaggctgcggcatcctgcaacctgatcctccagccaacatcaccgtgaccgccgtggccagaaatcccagatggctgtctgtgacctggcaggatccccacagctggaacagcagcttttaccggctgagattcgagctgcggtacagggccgagagaagcaagaccttcaccacctggatggtcaaggacctgcagcaccactgcgtgatccatgacgcttggagcggactgagacacgtggtgcagctgagagcccaagaagagtttggccaaggcgagtggagcgagtggtcacctgaagccatgggcacaccttggaccgagtctagatctccaccagccgagaacgaggtgtccacacctatgcaggccctgaccaccaacaaggacgacgacaacatcctgttccgggacagcgccaatgccacaagtctgcctgtgcaggatagctcctctgtgcctcttcctgcggccgcaaataatagctcaggggagatggatcctatcttactacctccgtgcctaaccatcagcattttgagttttttctctgtcgctctgttggtcatcttggcctgtgtgttatggaaaaaaaggattaagcctatcgtatggcccagtctccccgatcataagaagactctggaacatctttgtaagaaaccaagaaaaaatttaaatgtgagtttcaatcctgaaagtttcctggactgccagattcatagggtggatgacattcaagctagagatgaagtggaaggttttctgcaagatacgtttcctcagcaactagaagaatctgagaagcagaggcttggaggggatgtgcagagccccaactgcccatctgaggatgtagtcatcactccagaaagctttggaagagattcatccctcacatgcctggctgggaatgtcagtgcatgtgacgcccctattctctcctcttccaggtccctagactgcagggagagtggcaagaatgggcctcatgtgtaccaggacctcctgcttagccttgggactacaaacagcacgctgccccctccattttctctccaatctggaatcctgacattgaacccagttgctcagggtcagcccattcttacttccctgggatcaaatcaagaagaagcatatgtcaccatgtccagcttctaccaaaaccagtga

SEQ ID NO: 30 - DNA, 2490 bp, Artificial
  synthetic
atgctgaccctgcagacatggctggtgcaggccctgttcatcttcctgaccacagagagcacaggcgagctgctcgatccttgcggctacatctctcctgagagccctgtggtccagctgcacagcaatttcaccgccgtgtgcgtgctgaaagaaaagtgcatggactacttccacgtgaacgccaactacatcgtgtggaaaacgaaccacttcacgatccccaaagagcagtacaccatcatcaaccggaccgccagcagcgtgaccttcacagatatcgccagcctgaacatccagctgacctgcaacatcctgaccttcggccagctggaacagaacgtgtacggcatcacaatcatcagcggcctgcctccagagaagcccaagaacctgagctgcatcgtgaacgagggcaagaaaatgagatgcgagtgggacggcggcagagagacacacctggaaacaaacttcaccctgaagtccgagtgggccacacacaagttcgccgactgcaaggccaagagggatacccctaccagctgtaccgtggactacagcaccgtgtacttcgtgaacatcgaagtgtgggtcgaagccgagaacgccctgggcaaagtgaccagcgaccacatcaacttcgaccccgtgtacaaagtgaagcccaatcctcctcacaacctgagcgtgatcaacagcgaggaactgagcagcatcctgaagctgacatggacaaaccccagcatcaagtccgtgatcatcctcaagtacaacatccagtaccggaccaaggacgccagcacctggtcacagattcctccagaggataccgcctccaccagatccagcttcacagtgcaggacctgaagcctttcaccgagtacgtgttccggatcagatgcatgaaggaagatggcaaaggctactggagcgattggagcgaggaagccagcggcatcacctacgaggatagacctggctctgccggatctgctgctggctctggcgaattcgtggatgtgcctcctgaggaaccccagctgagctgcttcagaaagtcccctctgagcaacgtcgtgtgcgagtggggccctagaagcacacctagcctgacaacaaaggccgtgctgctcgtgcggaagttccagaatagccctgccgaggacttccaagagccttgccagtacagccaagagagccagaagttcagctgtcagctggccgtgcctgagggcgatagcagcttctacatcgtgtctatgtgcgtggccagcagcgtgggcagcaagtttagcaagacccagaccttccaaggctgcggcatcctgcaacctgatcctccagccaacatcaccgtgaccgccgtggccagaaatcccagatggctgtctgtgacctggcaggatccccacagctggaacagcagcttttaccggctgagattcgagctgcggtacagggccgagagaagcaagaccttcaccacctggatggtcaaggacctgcagcaccactgcgtgatccatgacgcttggagcggactgagacacgtggtgcagctgagagcccaagaagagtttggccaaggcgagtggagcgagtggtcacctgaagccatgggcacaccttggaccgagtctagatctccaccagccgagaacgaggtgtccacacctatgcaggccctgaccaccaacaaggacgacgacaacatcctgttccgggacagcgccaatgccacaagtctgcctgtgcaggatagctcctctgtgcctcttcctgcggccgcaaataatagctcaggggagatggatcctatcttactacctccgtgcctaaccatcagcattttgagttttttctctgtcgctctgttggtcatcttggcctgtgtgttatggaaaaaaaggattaagcctatcgtatggcccagtctccccgatcataagaagactctggaacatctttgtaagaaaccaagaaaaaatttaaatgtgagtttcaatcctgaaagtttcctggactgccagattcatagggtggatgacattcaagctagagatgaagtggaaggttttctgcaagatacgtttcctcagcaactagaagaatctgagaagcagaggcttggaggggatgtgcagagccccaactgcccatctgaggatgtagtcatcactccagaaagctttggaagagattcatccctcacatgcctggctgggaatgtcagtgcatgtgacgcccctattctctcctcttccaggtccctagactgcagggagagtggcaagaatgggcctcatgtgtaccaggacctcctgcttagccttgggactacaaacagcacgctgccccctccattttctctccaatctggaatcctgacattgaacccagttgctcagggtcagcccattcttacttccctgggatcaaatcaagaagaagcatatgtcaccatgtccagcttctaccaaaaccagtga

SEQ ID NO: 31 - DNA, 1737 bp, Artificial
  synthetic
atgctgagactgtacgtgctggttatgggcgtgtccgccttcacactgcagcctgcagctcatacaggcgccgctagaagctgcagattccggggcagacactacaagagagagttccggctggaaggcgagcccgtggctcttagatgtcctcaggtgccatattggctgtgggccagcgtgtcccctagaatcaatctgacctggcacaagaacgacagcgccagaacagtgcccggcgaggaagagacaagaatgtgggctcaagatggcgccctgtggcttctgcctgctctgcaagaggatagcggcacctacgtgtgcaccaccagaaacgccagctactgcgacaagatgagcatcgagctgcgggtgttcgagaacaccgacgcctttctgcccttcatcagctaccctcagatcctgacactgagcacctctggcgtgctcgtgtgtcctgatctgagcgagttcacccgggacaagaccgacgtgaagatccagtggtacaaggactccctgctgctggacaaggacaacgagaagttcctgagcgtgcggggcaccacacatctgctggtgcatgatgtggccctggaagatgccggctactacagatgcgtgctgacatttgcccacgagggccagcagtacaacatcaccagatctatcgagctgaggatcaagaagaagaaagaagagactatccccgtcatcatcagccctctgaaaaccatctctgccagcctgggcagcagactgacaatcccctgcaaggtgttcctcggcacaggcacccctctgaccacaatgctttggtggaccgccaacgacacccacatcgagtctgcttatcctggcggcagagtgacagagggccccagacaagagtacagcgagaacaatgagaactacatcgaggtgcccctgatcttcgaccccgtgaccagagaagatctgcacatggactttaagtgcgtggtgcataacaccctgagctttcagaccctgcggaccaccgtgaaagaggcggccgcaaataatagctcaggggagatggatcctatcttactacctccgtgcctaaccatcagcattttgagttttttctctgtcgctctgttggtcatcttggcctgtgtgttatggaaaaaaaggattaagcctatcgtatggcccagtctccccgatcataagaagactctggaacatctttgtaagaaaccaagaaaaaatttaaatgtgagtttcaatcctgaaagtttcctggactgccagattcatagggtggatgacattcaagctagagatgaagtggaaggttttctgcaagatacgtttcctcagcaactagaagaatctgagaagcagaggcttggaggggatgtgcagagccccaactgcccatctgaggatgtagtcatcactccagaaagctttggaagagattcatccctcacatgcctggctgggaatgtcagtgcatgtgacgcccctattctctcctcttccaggtccctagactgcagggagagtggcaagaatgggcctcatgtgtaccaggacctcctgcttagccttgggactacaaacagcacgctgccccctccattttctctccaatctggaatcctgacattgaacccagttgctcagggtcagcccattcttacttccctgggatcaaatcaagaagaagcatatgtcaccatgtccagcttctaccaaaaccagtga

SEQ ID NO: 32 - DNA, 1668 bp, Artificial
  synthetic
atgctgctgctggtcacatctctgctgctgtgcgagctgccccatcctgcctttctgctgatccccgagaagtccgacctgagaacagtggcccctgccagctctctgaacgttcgcttcgacagccggaccatgaacctgagctgggactgccaagagaacacaaccttcagcaagtgcttcctgaccgacaagaagaaccgggtcgtcgagcccagactgagcaacaatgagtgctcctgcaccttcagagagatctgcctgcacgagggcgtgacctttgaggtgcacgtgaacacaagccagcggggctttcagcagaagctgctgtaccccaatagcggcagagagggaaccgccgctcagaacttcagctgcttcatctacaacgccgacctcatgaactgcacctgggccagaggacctaccgctcctagagatgtgcagtacttcctgtacattcggaacagcaagcggcggagagaaatcaggtgcccctactacatccaagacagcggcacacacgtgggctgccacctggataatctgtctggcctgaccagccggaactacttcctggtcaatggcaccagccgcgagatcggcatccagttctttgacagcctgctggacaccaagaagatcgagcggttcaaccctcctagcaacgtgaccgtgcggtgcaacaccacacattgtctcgtgcggtggaagcagccccggacataccagaagctgagctacctggacttccagtaccagctggacgtgcaccggaagaatacccagcctggcaccgagaacctgctgatcaatgtgtccggcgacctggaaaaccggtacaacttccctagcagcgagcccagggccaagcacagcgtgaaaattagagccgccgacgtgcggatcctgaactggtcatcttggagcgaggccatcgagttcggctctgatgacggagcggccgcaaataatagctcaggggagatggatcctatcttactacctccgtgcctaaccatcagcattttgagttttttctctgtcgctctgttggtcatcttggcctgtgtgttatggaaaaaaaggattaagcctatcgtatggcccagtctccccgatcataagaagactctggaacatctttgtaagaaaccaagaaaaaatttaaatgtgagtttcaatcctgaaagtttcctggactgccagattcatagggtggatgacattcaagctagagatgaagtggaaggttttctgcaagatacgtttcctcagcaactagaagaatctgagaagcagaggcttggaggggatgtgcagagccccaactgcccatctgaggatgtagtcatcactccagaaagctttggaagagattcatccctcacatgcctggctgggaatgtcagtgcatgtgacgcccctattctctcctcttccaggtccctagactgcagggagagtggcaagaatgggcctcatgtgtaccaggacctcctgcttagccttgggactacaaacagcacgctgccccctccattttctctccaatctggaatcctgacattgaacccagttgctcagggtcagcccattcttacttccctgggatcaaatcaagaagaagcatatgtcaccatgtccagcttctaccaaaaccagtga

SEQ ID NO: 33 - DNA, 2037 bp, Artificial
  synthetic
atggtgctggctcaaggactgctttctatggccctgctggccctgtgttgggagagaagtcttgccggcgctgaagagacaatccctctgcagaccctgcggtgctacaacgactacaccagccacatcacctgtagatgggccgacacacaggacgcccagagactcgtgaatgtgaccctgatcagaagagtgaacgaggacctgctggaacccgtgtcctgtgacctgagcgacgatatgccttggagcgcctgtcctcatcctagatgtgtgcctcggagatgcgtgatcccttgccagagcttcgtggtcaccgacgtggactacttcagcttccagcctgacagacccctgggcaccagactgacagtgacactgacacagcacgtgcagcctccagagcctagagatctccagatttctaccgaccaggaccacttcctgctgacttggagtgtggctctgggcagccctcagtctcattggcttagccctggcgatctggaattcgaggtggtgtacaagcggctgcaggacagctgggaagatgccgccattctgctgagcaatacctctcaggccacactgggccccgaacacctgatgccttctagcacatacgtggccagagtgcggacaagactggcccctggatctagactgagcggcagaccttctaagtggtcccctgaagtgtgctgggactctcagcctggggatgaagcccagcctcagaacctggaatgcttctttgatggcgccgcagtgctgagctgctcttgggaagtgcggaaagaggtggccagcagcgttagcttcggcctgttctacaagccctctcctgacgccggcgaagaggaatgttctcccgtgctgagagaaggcctgggaagcctgcacaccagacaccactgtcagatccccgtgcctgatcctgccacacacggccagtatatcgtgtccgtgcagccaagaagggccgagaagcacatcaagtccagcgtgaacatccagatggccccacctagcctgaacgtgaccaaggacggcgacagctacagcctgagatgggagacaatgaagatgcgctacgagcacatcgaccacaccttcgagatccagtaccggaaggacaccgccacatggaaggacagcaagaccgagacactgcagaacgcccacagcatggctctgcctgctctggaacctagcaccagatactgggctagagtccgcgtgcggaccagcagaacaggctacaatggcatttggagcgagtggagcgaagccagaagctgggataccgagagcgtgttgcctatgtgggcggccgcaaataatagctcaggggagatggatcctatcttactacctccgtgcctaaccatcagcattttgagttttttctctgtcgctctgttggtcatcttggcctgtgtgttatggaaaaaaaggattaagcctatcgtatggcccagtctccccgatcataagaagactctggaacatctttgtaagaaaccaagaaaaaatttaaatgtgagtttcaatcctgaaagtttcctggactgccagattcatagggtggatgacattcaagctagagatgaagtggaaggttttctgcaagatacgtttcctcagcaactagaagaatctgagaagcagaggcttggaggggatgtgcagagccccaactgcccatctgaggatgtagtcatcactccagaaagctttggaagagattcatccctcacatgcctggctgggaatgtcagtgcatgtgacgcccctattctctcctcttccaggtccctagactgcagggagagtggcaagaatgggcctcatgtgtaccaggacctcctgcttagccttgggactacaaacagcacgctgccccctccattttctctccaatctggaatcctgacattgaacccagttgctcagggtcagcccattcttacttccctgggatcaaatcaagaagaagcatatgtcaccatgtccagcttctaccaaaaccagtga

SEQ ID NO: 34 - protein, 17 aa, Bombyx mori
MMRPIVLVLLFATSALA

SEQ ID NO: 35 - protein, 220 aa, Homo sapiens
MLRLLLALNLFPSIQVTGNKILVKQSPMLVAYDNAVNLSCKYSYNLFSREFRASLHKGLDSAVEVCVVYGNYSQQLQVYSKTGFNCDGKLGNESVTFYLQNLYVNQTDIYFCKIEVMYPPPYLDNEKSNGTIIHVKGKHLCPSPLFPGPSKPFWVLVVVGGVLACYSLLVTVAFIIFWVRSKRSRLLHSDYMNMTPRRPGPTRKHYQPYAPPRDFAAYRS

SEQ ID NO: 36 - protein, 704 aa, Artificial
  synthetic
MLTLQTWLVQALFIFLTTESTGELLDPCGYISPESPVVQLHSNFTAVCVLKEKCMDYFHVNANYIVWKTNHFTIPKEQYTIINRTASSVTFTDIASLNIQLTCNILTFGQLEQNVYGITIISGLPPEKPKNLSCIVNEGKKMRCEWDGGRETHLETNFTLKSEWATHKFADCKAKRDTPTSCTVDYSTVYFVNIEVWVEAENALGKVTSDHINFDPVYKVKPNPPHNLSVINSEELSSILKLTWTNPSIKSVIILKYNIQYRTKDASTWSQIPPEDTASTRSSFTVQDLKPFTEYVFRIRCMKEDGKGYWSDWSEEASGITYEDRPGSAGSAAGSGEFVDVPPEEPQLSCFRKSPLSNVVCEWGPRSTPSLTTKAVLLVRKFQNSPAEDFQEPCQYSQESQKFSCQLAVPEGDSSFYIVSMCVASSVGSKFSKTQTFQGCGILQPDPPANITVTAVARNPRWLSVTWQDPHSWNSSFYRLRFELRYRAERSKTFTTWMVKDLQHHCVIHDAWSGLRHVVQLRAQEEFGQGEWSEWSPEAMGTPWTESRSPPAENEVSTPMQALTTNKDDDNILFRDSANATSLPVQDSSSVPLPAAAIEVMYPPPYLDNEKSNGTIIHVKGKHLCPSPLFPGPSKPFWVLVVVGGVLACYSLLVTVAFIIFWVRSKRSRLLHSDYMNMPPRRPGPTRKHYQPYAPPRDFAAYRS